European Patent Application EP 4 488 290 A1, published January 8, 2025. Title: 티올 반응성 에디티브를 이용한 항체-약물 컨쥬게이트의 제조 수율을 높이는 방법. Applicant: 앱티스 주식회사. Application KR. The sequence listing filed with the application follows.

SEQUENCE LISTING (82 sequences)

SEQ ID NO: 1 - protein, 17 aa, synthetic construct
GPSVFLFPPKPKDTLMI

SEQ ID NO: 2 - protein, 17 aa, synthetic construct
RGNCAYHKGQIIWCTYH

SEQ ID NO: 3 - protein, 17 aa, synthetic construct
RGNCAYHKGQIVWCTYH

SEQ ID NO: 4 - protein, 17 aa, synthetic construct
RGNCAYHKGQVVWCTYH

SEQ ID NO: 5 - protein, 17 aa, synthetic construct
RGNCAYHKGQAVWCTYH

SEQ ID NO: 6 - protein, 17 aa, synthetic construct
RGNCAYHKGQLLWCTYH

SEQ ID NO: 7 - protein, 17 aa, synthetic construct
RGNCAYHKGQLIWCTYH

SEQ ID NO: 8 - protein, 13 aa, synthetic construct
DCAYHKGQIVWCT

SEQ ID NO: 9 - protein, 13 aa, synthetic construct
DCAYHKGQVVWCT

SEQ ID NO: 10 - protein, 13 aa, synthetic construct
DCAYHKGQAVWCT

SEQ ID NO: 11 - protein, 17 aa, synthetic construct
RGNCAYHKSQIIWCTYH

SEQ ID NO: 12 - protein, 17 aa, synthetic construct
RGNCAYHKNQIIWCTYH

SEQ ID NO: 13 - protein, 17 aa, synthetic construct
RGNCAYHKDQIIWCTYH

SEQ ID NO: 14 - protein, 17 aa, synthetic construct
RGNCAYHKQQIIWCTYH

SEQ ID NO: 15 - protein, 17 aa, synthetic construct
RGNCAYHKEQIIWCTYH

SEQ ID NO: 16 - protein, 17 aa, synthetic construct
RGNCAYHKFQIIWCTYH

SEQ ID NO: 17 - protein, 17 aa, synthetic construct
RGNCAYHKYQIIWCTYH

SEQ ID NO: 18 - protein, 17 aa, synthetic construct
RGNCAYHKWQIIWCTYH

SEQ ID NO: 19 - protein, 17 aa, synthetic construct
RGNCAYHKHQIIWCTYH

SEQ ID NO: 20 - protein, 17 aa, synthetic construct
RGNCAYHKTQIIWCTYH

SEQ ID NO: 21 - protein, 17 aa, synthetic construct
RGNCAYHKLQIIWCTYH

SEQ ID NO: 22 - protein, 11 aa, synthetic construct
CAYHKLQIVWC

SEQ ID NO: 23 - protein, 11 aa, synthetic construct
CAYHKLQLIWC

SEQ ID NO: 24 - protein, 11 aa, synthetic construct
CAYHKSQIVWC

SEQ ID NO: 25 - protein, 17 aa, synthetic construct
RGNCAYHKGQLVFCTYH

SEQ ID NO: 26 - protein, 17 aa, synthetic construct
RGNCAYHKGQQVWCTYH

SEQ ID NO: 27 - protein, 17 aa, synthetic construct
RGNCAYHKGQEVWCTYH

SEQ ID NO: 28 - protein, 11 aa, synthetic construct
CAYHKGQLVWC

SEQ ID NO: 29 - protein, 17 aa, synthetic construct
RGNCAYHKAQLVWCTYH

SEQ ID NO: 30 - protein, 17 aa, synthetic construct
RGNCAYHKVQLVWCTYH

SEQ ID NO: 31 - protein, 17 aa, synthetic construct
RGNCAYHKLQLVWCTYH

SEQ ID NO: 32 - protein, 17 aa, synthetic construct
RGNCAYHKIQLVWCTYH

SEQ ID NO: 33 - protein, 17 aa, synthetic construct
RGNCAYHKSQLVWCTYH

SEQ ID NO: 34 - protein, 17 aa, synthetic construct
RGNCAYHKTQLVWCTYH

SEQ ID NO: 35 - protein, 17 aa, synthetic construct
RGNCAYHKNQLVWCTYH

SEQ ID NO: 36 - protein, 17 aa, synthetic construct
RGNCAYHKDQLVWCTYH

SEQ ID NO: 37 - protein, 17 aa, synthetic construct
RGNCAYHKQQLVWCTYH

SEQ ID NO: 38 - protein, 17 aa, synthetic construct
RGNCAYHKEQLVWCTYH

SEQ ID NO: 39 - protein, 17 aa, synthetic construct
RGNCAYHKFQLVWCTYH

SEQ ID NO: 40 - protein, 17 aa, synthetic construct
RGNCAYHKRQLVWCTYH

SEQ ID NO: 41 - protein, 17 aa, synthetic construct
RGNCAYHKHQLVWCTYH

SEQ ID NO: 42 - protein, 17 aa, synthetic construct
RGNCAYHKWQLVWCTYH

SEQ ID NO: 43 - protein, 17 aa, synthetic construct
RGNCAYHKYQLVWCTYH

SEQ ID NO: 44 - protein, 17 aa, synthetic construct
RGNCAYFKGQLVWCTYH

SEQ ID NO: 45 - protein, 17 aa, synthetic construct
RGNCAYYKGQLVWCTYH

SEQ ID NO: 46 - protein, 17 aa, synthetic construct
RGNCAYWKGQLVWCTYH

SEQ ID NO: 47 - protein, 17 aa, synthetic construct
RGNCAYRKGQLVWCTYH

SEQ ID NO: 48 - protein, 17 aa, synthetic construct
RGNCAYGKGQLVWCTYH

SEQ ID NO: 49 - protein, 12 aa, synthetic construct
DCAYHKGQLVWC

SEQ ID NO: 50 - protein, 12 aa, synthetic construct
NCAYHKGQLVWC

SEQ ID NO: 51 - protein, 12 aa, synthetic construct
CAYHKGQLVWCT

SEQ ID NO: 52 - protein, 11 aa, synthetic construct
CAYHKSQLVWC

SEQ ID NO: 53 - protein, 16 aa, synthetic construct
GNCAYHKGQIIWCTYH

SEQ ID NO: 54 - protein, 17 aa, synthetic construct
RGNCAYHEGQIIWCTYH

SEQ ID NO: 55 - protein, 17 aa, synthetic construct
GPDCAYHRGELVWCTFH

SEQ ID NO: 56 - protein, 13 aa, synthetic construct
  source 1..13: note = Fc binding peptide
  SITE 6: note = wherein X represents diaminopropionic acid
DCAWHXGELVWCT

SEQ ID NO: 57 - protein, 13 aa, synthetic construct
  source 1..13: note = Fc binding peptide
  SITE 6: note = wherein X represents diaminobutyric acid
DCAWHXGELVWCT

SEQ ID NO: 58 - protein, 13 aa, synthetic construct
  SITE 6: note = wherein X represents Ornithine residue
DCAWHXGELVWCT

SEQ ID NO: 59 - protein, 13 aa, synthetic construct
DCAWHKGELVWCT

SEQ ID NO: 60 - protein, 13 aa, synthetic construct
DCAWHLGELVWCT

SEQ ID NO: 61 - protein, 17 aa, synthetic construct
RGNCAYHRGKLVWCTYH

SEQ ID NO: 62 - protein, 17 aa, synthetic construct
RGNCAYHKGQLVWCTYH

SEQ ID NO: 63 - protein, 17 aa, synthetic construct
  SITE 8: note = wherein X represents diaminopropionic acid.
GPDCAYHXGELVWCTFH

SEQ ID NO: 64 - protein, 17 aa, synthetic construct
  SITE 8: note = X represents diaminobutyric acid.
GPDCAYHXGELVWCTFH

SEQ ID NO: 65 - protein, 17 aa, synthetic construct
  SITE 8: note = X represents ornithine residue.
GPDCAYHXGELVWCTFH

SEQ ID NO: 66 - protein, 17 aa, synthetic construct
GPDCAYHKGELVWCTFH

SEQ ID NO: 67 - protein, 17 aa, synthetic construct
  SITE 10: note = X represents diaminopropionic acid.
GPDCAYHRGXLVWCTFH

SEQ ID NO: 68 - protein, 17 aa, synthetic construct
  SITE 10: note = X represents diaminobutyric acid.
GPDCAYHRGXLVWCTFH

SEQ ID NO: 69 - protein, 17 aa, synthetic construct
  SITE 10: note = X represents ornithine residue.
GPDCAYHRGXLVWCTFH

SEQ ID NO: 70 - protein, 17 aa, synthetic construct
GPDCAYHRGKLVWCTFH

SEQ ID NO: 71 - protein, 13 aa, synthetic construct
  SITE 1: note = wherein X represents any amino acid residue other than cysteine residue.
  SITE 3..4: note = wherein X each independently represents any amino acid residue other than cysteine residue.
  SITE 6: note = wherein X represents luecine, diaminopropionic acid, diaminobytyric acid, ornithine, or lysine residue
  SITE 8: note = wherein X represents glutamic acid or asparagine residue
  SITE 11: note = wherein X represents tryptophan, naphthylalanine, or phenylalanine residue
  SITE 13: note = wherein X represents any amino acid residue other than cysteine residue.
XCXXHXGXLVXCX

SEQ ID NO: 72 - protein, 14 aa, synthetic construct
  source 1..14: note = Fc binding peptide
  SITE 1: note = wherein X represents any amino acid residue other than cysteine residue.
  SITE 3..4: note = wherein X each independently represents any amino acid residue other than cysteine residue.
  SITE 6: note = wherein X represents cysteine, luecine, diaminopropionic acid, diaminobytyric acid, ornithine, or lysine residue
  SITE 8: note = wherein X represents glutamic acid or asparagine residue
  SITE 11: note = wherein X represents Tryptophan, naphthylalanine, or phenylalanine residue
  SITE 13..14: note = wherein X each independently represents any amino acid residue other than cysteine residue.
XCXXHXGXLVXCXX

SEQ ID NO: 73 - protein, 15 aa, synthetic construct
  source 1..15: note = Fc binding peptide
  SITE 1: note = wherein X represents any amino acid residue other than cysteine residue
  SITE 3..4: note = wherein X each independently represents any amino acid residue other than cysteine residue
  SITE 6: note = wherein X represents cysteine, luecine, diaminopropionic acid, diaminobytyric acid, ornithine, or lysine residue
  SITE 8: note = wherein X represents glutamic acid or asparagine residue
  SITE 11: note = wherein X represents Tryptophan, naphthylalanine, or phenylalanine residue
  SITE 13..15: note = wherein X each independently represents any amino acid residue other than cysteine residue.
XCXXHXGXLVXCXXX

SEQ ID NO: 74 - protein, 14 aa, synthetic construct
  source 1..14: note = Fc binding peptide
  SITE 1..2: note = wherein X each independently represents any amino acid residue other than cysteine residue.
  SITE 4..5: note = wherein X each independently represents any amino acid residue other than cysteine residue.
  SITE 7: note = wherein X represents cysteine, luecine, diaminopropionic acid, diaminobytyric acid, ornithine, or lysine residue
  SITE 9: note = wherein X represents glutamic acid or asparagine residue.
  SITE 12: note = wherein X represents Tryptophan, naphthylalanine, or phenylalanine residue.
XXCXXHXGXLVXCX

SEQ ID NO: 75 - protein, 15 aa, synthetic construct
  source 1..15: note = Fc binding peptide
  SITE 1..2: note = wherein X each independently represents any amino acid residue other than cysteine residue.
  SITE 4..5: note = wherein X each independently represents any amino acid residue other than cysteine residue.
  SITE 7: note = wherein X represents cysteine, luecine, diaminopropionic acid, diaminobytyric acid, ornithine, or lysine residue.
  SITE 9: note = wherein X represents glutamic acid or asparagine residue.
  SITE 12: note = wherein X represents Tryptophan, naphthylalanine, or phenylalanine residue.
  SITE 14..15: note = wherein X each independently represents any amino acid residue other than cysteine residue.
XXCXXHXGXLVXCXX

SEQ ID NO: 76 - protein, 16 aa, synthetic construct
  SITE 1..2: note = wherein X each independently represents any amino acid residue other than cysteine residue.
  SITE 4..5: note = wherein X each independently represents any amino acid residue other than cysteine residue.
  SITE 7: note = wherein X represents cysteine, luecine, diaminopropionic acid, diaminobytyric acid, ornithine, or lysine residue
  SITE 9: note = wherein X represents glutamic acid or asparagine residue
  SITE 12: note = wherein X represents Tryptophan, naphthylalanine, or phenylalanine residue
  SITE 14..16: note = wherein X each independently represents any amino acid residue other than cysteine residue.
XXCXXHXGXLVXCXXX

SEQ ID NO: 77 - protein, 15 aa, synthetic construct
  source 1..15: note = Fc binding peptide
  SITE 1..3: note = wherein X each independently represents any amino acid residue other than cysteine residue.
  SITE 5..6: note = wherein X each independently represents any amino acid residue other than cysteine residue.
  SITE 8: note = wherein X represents cysteine, luecine, diaminopropionic acid, diaminobytyric acid, ornithine, or lysine residue.
  SITE 10: note = wherein X represents glutamic acid or asparagine residue.
  SITE 13: note = wherein X represents Tryptophan, naphthylalanine, or phenylalanine residue.
  SITE 15: note = wherein X represents any amino acid residue other than cysteine residue.
XXXCXXHXGXLVXCX

SEQ ID NO: 78 - protein, 16 aa, synthetic construct
  source 1..16: note = Fc binding peptide
  SITE 1..3: note = wherein X each independently represents any amino acid residue other than cysteine residue.
  SITE 5..6: note = wherein X each independently represents any amino acid residue other than cysteine residue.
  SITE 8: note = wherein X represents cysteine, luecine, diaminopropionic acid, diaminobytyric acid, ornithine, or lysine residue.
  SITE 10: note = wherein X represents glutamic acid or asparagine residue.
  SITE 13: note = wherein X represents Tryptophan, naphthylalanine, or phenylalanine residue.
  SITE 15..16: note = wherein X each independently represents any amino acid residue other than cysteine residue.
XXXCXXHXGXLVXCXX

SEQ ID NO: 79 - protein, 17 aa, synthetic construct
  source 1..17: note = Fc binding peptide
  SITE 1..3: note = wherein X each independently represents any amino acid residue other than cysteine residue.
  SITE 5..6: note = wherein X each independently represents any amino acid residue other than cysteine residue.
  SITE 8: note = wherein X represents cysteine, luecine, diaminopropionic acid, diaminobytyric acid, ornithine, or lysine residue.
  SITE 10: note = wherein X represents glutamic acid or asparagine residue.
  SITE 13: note = wherein X represents Tryptophan, naphthylalanine, or phenylalanine residue
  SITE 15..17: note = wherein X each independently represents any amino acid residue other than cysteine residue.
XXXCXXHXGXLVXCXXX

SEQ ID NO: 80 - protein, 13 aa, synthetic construct
  source 1..13: note = Fc binding peptide
  SITE 3..4: note = wherein X each independently represents any amino acid residue other than cysteine residue.
  SITE 6: note = wherein X represents cysteine, luecine, diaminopropionic acid, diaminobytyric acid, ornithine, or lysine residue
  SITE 8: note = wherein X represents glutamic acid or asparagine residue.
  SITE 11: note = wherein X represents Tryptophan, naphthylalanine, or phenylalanine residue.
DCXXHXGXLVXCT

SEQ ID NO: 81 - protein, 220 aa, synthetic construct
DIVMTQSPLSLPVTPGEPASISCKSSQTLLNSGNQKNYLTWYLQKPGQSPQLLIYWASTGESGVPDRFSGSGSGTDFTLKISRVEAEDVGVYYCQNAYFYPFTFGGGTKVEIKRTVAAPSVFIFPPSDEQLKSGTASVVCLLNNFYPREAKVQWKVDNALQSGNSQESVTEQDSKDSTYSLSSTLTLSKADYEKHKVYACEVTHQGLSSPVTKSFNRGEC

SEQ ID NO: 82 - protein, 448 aa, synthetic construct
QVQLVESGGGVVQPGRSLRLSCAASGFSLTTYGVHWVRQAPGKGLEWVAVIWAGGSTNYNSALMSRFTISRDNSKNTLYLQMNSLRAEDTAVYYCARAAYYGNGLDYWGQGTMVTVSSASTKGPSVFPLAPSSKSTSGGTAALGCLVKDYFPEPVTVSWNSGALTSGVHTFPAVLQSSGLYSLSSVVTVPSSSLGTQTYICNVNHKPSNTKVDKRVEPKSCDKTHTCPPCPAPELLGGPSVFLFPPKPKDTLMISRTPEVTCVVVDVSHEDPEVKFNWYVDGVEVHNAKTKPREEQYNSTYRVVSVLTVLHQDWLNGKEYKCKVSNKALPAPIEKTISKAKGQPREPQVYTLPPSRDELTKNQVSLTCLVKGFYPSDIAVEWESNGQPENNYKTTPPVLDSDGSFFLYSKLTVDKSRWQQGNVFSCSVMHEALHNHYTQKSLSLSPGK